European Patent Specification EP 2 894 165 B1, published January 4, 2023. Title: METHODS AND COMPOSITIONS FOR TREATING COMPLEMENT-ASSOCIATED DISORDERS. Applicant: ALEXION PHARMACEUTICALS, INC. The sequence listing filed with the application follows.

SEQUENCE LISTING (26 sequences)

SEQ ID NO: 1 - protein, 1676 aa, Homo sapiens
MGLLGILCFLIFLGKTWGQEQTYVISAPKIFRVGASENIVIQVYGYTEAFDATISIKSYPDKKFSYSSGHVHLSSENKFQNSAILTIQPKQLPGGQNPVSYVYLEVVSKHFSKSKRMPITYDNGFLFIHTDKPVYTPDQSVKVRVYSLNDDLKPAKRETVLTFIDPEGSEVDMVEEIDHIGIISFPDFKIPSNPRYGMWTIKAKYKEDFSTTGTAYFEVKEYVLPHFSVSIEPEYNFIGYKNFKNFEITIKARYFYNKVVTEADVYITFGIREDLKDDQKEMMQTAMQNTMLINGIAQVTFDSETAVKELSYYSLEDLNNKYLYIAVTVIESTGGFSEEAEIPGIKYVLSPYKLNLVATPLFLKPGIPYPIKVQVKDSLDQLVGGVPVILNAQTIDVNQETSDLDPSKSVTRVDDGVASFVLNLPSGVTVLEFNVKTDAPDLPEENQAREGYRAIAYSSLSQSYLYIDWTDNHKALLVGEHLNIIVTPKSPYIDKITHYNYLILSKGKIIHFGTREKFSDASYQSINIPVTQNMVPSSRLLVYYIVTGEQTAELVSDSVWLNIEEKCGNQLQVHLSPDADAYSPGQTVSLNMATGMDSWVALAAVDSAVYGVQRGAKKPLERVFQFLEKSDLGCGAGGGLNNANVFHLAGLTFLTNANADDSQENDEPCKEILRPRRTLQKKIEEIAAKYKHSVVKKCCYDGACVNNDETCEQRAARISLGPRCIKAFTECCVVASQLRANISHKDMQLGRLHMKTLLPVSKPEIRSYFPESWLWEVHLVPRRKQLQFALPDSLTTWEIQGIGISNTGICVADTVKAKVFKDVFLEMNIPYSVVRGEQIQLKGTVYNYRTSGMQFCVKMSAVEGICTSESPVIDHQGTKSSKCVRQKVEGSSSHLVTFTVLPLEIGLHNINFSLETWFGKEILVKTLRVVPEGVKRESYSGVTLDPRGIYGTISRRKEFPYRIPLDLVPKTEIKRILSVKGLLVGEILSAVLSQEGINILTHLPKGSAEAELMSVVPVFYVFHYLETGNHWNIFHSDPLIEKQKLKKKLKEGMLSIMSYRNADYSYSVWKGGSASTWLTAFALRVLGQVNKYVEQNQNSICNSLLWLVENYQLDNGSFKENSQYQPIKLQGTLPVEARENSLYLTAFTVIGIRKAFDICPLVKIDTALIKADNFLLENTLPAQSTFTLAISAYALSLGDKTHPQFRSIVSALKREALVKGNPPIYRFWKDNLQHKDSSVPNTGTARMVETTAYALLTSLNLKDINYVNPVIKWLSEEQRYGGGFYSTQDTINAIEGLTEYSLLVKQLRLSMDIDVSYKHKGALHNYKMTDKNFLGRPVEVLLNDDLIVSTGFGSGLATVHVTTVVHKTSTSEEVCSFYLKIDTQDIEASHYRGYGNSDYKRIVACASYKPSREESSSGSSHAVMDISLPTGISANEEDLKALVEGVDQLFTDYQIKDGHVILQLNSIPSSDFLCVRFRIFELFEVGFLSPATFTVYEYHRPDKQCTMFYSTSNIKIQKVCEGAACKCVEADCGQMQEELDLTISAETRKQTACKPEIAYAYKVSITSITVENVFVKYKATLLDIYKTGEAVAEKDSEITFIKKVTCTNAELVKGRQYLIMGKEALQIKYNFSFRYIYPLDSLTWIEYWPRDTTCSSCQAFLANLDEFAEDIFLNGC

SEQ ID NO: 2 - protein, 1658 aa, Homo sapiens
QEQTYVISAPKIFRVGASENIVIQVYGYTEAFDATISIKSYPDKKFSYSSGHVHLSSENKFQNSAILTIQPKQLPGGQNPVSYVYLEVVSKHFSKSKRMPITYDNGFLFIHTDKPVYTPDQSVKVRVYSLNDDLKPAKRETVLTFIDPEGSEVDMVEEIDHIGIISFPDFKIPSNPRYGMWTIKAKYKEDFSTTGTAYFEVKEYVLPHFSVSIEPEYNFIGYKNFKNFEITIKARYFYNKVVTEADVYITFGIREDLKDDQKEMMQTAMQNTMLINGIAQVTFDSETAVKELSYYSLEDLNNKYLYIAVTVIESTGGFSEEAEIPGIKYVLSPYKLNLVATPLFLKPGIPYPIKVQVKDSLDQLVGGVPVILNAQTIDVNQETSDLDPSKSVTRVDDGVASFVLNLPSGVTVLEFNVKTDAPDLPEENQAREGYRAIAYSSLSQSYLYIDWTDNHKALLVGEHLNIIVTPKSPYIDKITHYNYLILSKGKIIHFGTREKFSDASYQSINIPVTQNMVPSSRLLVYYIVTGEQTAELVSDSVWLNIEEKCGNQLQVHLSPDADAYSPGQTVSLNMATGMDSWVALAAVDSAVYGVQRGAKKPLERVFQFLEKSDLGCGAGGGLNNANVFHLAGLTFLTNANADDSQENDEPCKEILRPRRTLQKKIEEIAAKYKHSVVKKCCYDGACVNNDETCEQRAARISLGPRCIKAFTECCVVASQLRANISHKDMQLGRLHMKTLLPVSKPEIRSYFPESWLWEVHLVPRRKQLQFALPDSLTTWEIQGIGISNTGICVADTVKAKVFKDVFLEMNIPYSVVRGEQIQLKGTVYNYRTSGMQFCVKMSAVEGICTSESPVIDHQGTKSSKCVRQKVEGSSSHLVTFTVLPLEIGLHNINFSLETWFGKEILVKTLRVVPEGVKRESYSGVTLDPRGIYGTISRRKEFPYRIPLDLVPKTEIKRILSVKGLLVGEILSAVLSQEGINILTHLPKGSAEAELMSVVPVFYVFHYLETGNHWNIFHSDPLIEKQKLKKKLKEGMLSIMSYRNADYSYSVWKGGSASTWLTAFALRVLGQVNKYVEQNQNSICNSLLWLVENYQLDNGSFKENSQYQPIKLQGTLPVEARENSLYLTAFTVIGIRKAFDICPLVKIDTALIKADNFLLENTLPAQSTFTLAISAYALSLGDKTHPQFRSIVSALKREALVKGNPPIYRFWKDNLQHKDSSVPNTGTARMVETTAYALLTSLNLKDINYVNPVIKWLSEEQRYGGGFYSTQDTINAIEGLTEYSLLVKQLRLSMDIDVSYKHKGALHNYKMTDKNFLGRPVEVLLNDDLIVSTGFGSGLATVHVTTVVHKTSTSEEVCSFYLKIDTQDIEASHYRGYGNSDYKRIVACASYKPSREESSSGSSHAVMDISLPTGISANEEDLKALVEGVDQLFTDYQIKDGHVILQLNSIPSSDFLCVRFRIFELFEVGFLSPATFTVYEYHRPDKQCTMFYSTSNIKIQKVCEGAACKCVEADCGQMQEELDLTISAETRKQTACKPEIAYAYKVSITSITVENVFVKYKATLLDIYKTGEAVAEKDSEITFIKKVTCTNAELVKGRQYLIMGKEALQIKYNFSFRYIYPLDSLTWIEYWPRDTTCSSCQAFLANLDEFAEDIFLNGC

SEQ ID NO: 3 - protein, 999 aa, Homo sapiens
TLQKKIEEIAAKYKHSVVKKCCYDGACVNNDETCEQRAARISLGPRCIKAFTECCVVASQLRANISHKDMQLGRLHMKTLLPVSKPEIRSYFPESWLWEVHLVPRRKQLQFALPDSLTTWEIQGIGISNTGICVADTVKAKVFKDVFLEMNIPYSVVRGEQIQLKGTVYNYRTSGMQFCVKMSAVEGICTSESPVIDHQGTKSSKCVRQKVEGSSSHLVTFTVLPLEIGLHNINFSLETWFGKEILVKTLRVVPEGVKRESYSGVTLDPRGIYGTISRRKEFPYRIPLDLVPKTEIKRILSVKGLLVGEILSAVLSQEGINILTHLPKGSAEAELMSVVPVFYVFHYLETGNHWNIFHSDPLIEKQKLKKKLKEGMLSIMSYRNADYSYSVWKGGSASTWLTAFALRVLGQVNKYVEQNQNSICNSLLWLVENYQLDNGSFKENSQYQPIKLQGTLPVEARENSLYLTAFTVIGIRKAFDICPLVKIDTALIKADNFLLENTLPAQSTFTLAISAYALSLGDKTHPQFRSIVSALKREALVKGNPPIYRFWKDNLQHKDSSVPNTGTARMVETTAYALLTSLNLKDINYVNPVIKWLSEEQRYGGGFYSTQDTINAIEGLTEYSLLVKQLRLSMDIDVSYKHKGALHNYKMTDKNFLGRPVEVLLNDDLIVSTGFGSGLATVHVTTVVHKTSTSEEVCSFYLKIDTQDIEASHYRGYGNSDYKRIVACASYKPSREESSSGSSHAVMDISLPTGISANEEDLKALVEGVDQLFTDYQIKDGHVILQLNSIPSSDFLCVRFRIFELFEVGFLSPATFTVYEYHRPDKQCTMFYSTSNIKIQKVCEGAACKCVEADCGQMQEELDLTISAETRKQTACKPEIAYAYKVSITSITVENVFVKYKATLLDIYKTGEAVAEKDSEITFIKKVTCTNAELVKGRQYLIMGKEALQIKYNFSFRYIYPLDSLTWIEYWPRDTTCSSCQAFLANLDEFAEDIFLNGC

SEQ ID NO: 4 - protein, 655 aa, Homo sapiens
QEQTYVISAPKIFRVGASENIVIQVYGYTEAFDATISIKSYPDKKFSYSSGHVHLSSENKFQNSAILTIQPKQLPGGQNPVSYVYLEVVSKHFSKSKRMPITYDNGFLFIHTDKPVYTPDQSVKVRVYSLNDDLKPAKRETVLTFIDPEGSEVDMVEEIDHIGIISFPDFKIPSNPRYGMWTIKAKYKEDFSTTGTAYFEVKEYVLPHFSVSIEPEYNFIGYKNFKNFEITIKARYFYNKVVTEADVYITFGIREDLKDDQKEMMQTAMQNTMLINGIAQVTFDSETAVKELSYYSLEDLNNKYLYIAVTVIESTGGFSEEAEIPGIKYVLSPYKLNLVATPLFLKPGIPYPIKVQVKDSLDQLVGGVPVILNAQTIDVNQETSDLDPSKSVTRVDDGVASFVLNLPSGVTVLEFNVKTDAPDLPEENQAREGYRAIAYSSLSQSYLYIDWTDNHKALLVGEHLNIIVTPKSPYIDKITHYNYLILSKGKIIHFGTREKFSDASYQSINIPVTQNMVPSSRLLVYYIVTGEQTAELVSDSVWLNIEEKCGNQLQVHLSPDADAYSPGQTVSLNMATGMDSWVALAAVDSAVYGVQRGAKKPLERVFQFLEKSDLGCGAGGGLNNANVFHLAGLTFLTNANADDSQENDEPCKEIL

SEQ ID NO: 5 - protein, 21 aa, Homo sapiens
VIDHQGTKSSKCVRQKVEGSS

SEQ ID NO: 6 - protein, 5 aa, Homo sapiens
KSSKC

SEQ ID NO: 7 - protein, 127 aa, Homo sapiens
NFSLETWFGKEILVKTLRVVPEGVKRESYSGVTLDPRGIYGTISRRKEFPYRIPLDLVPKTEIKRILSVKGLLVGEILSAVLSQEGINILTHLPKGSAEAELMSVVPVFYVFHYLETGNHWNIFHSD

SEQ ID NO: 8 - protein, 200 aa, Homo sapiens
SESPVIDHQGTKSSKCVRQKVEGSSSHLVTFTVLPLEIGLHNINFSLETWFGKEILVKTLRVVPEGVKRESYSGVTLDPRGIYGTISRRKEFPYRIPLDLVPKTEIKRILSVKGLLVGEILSAVLSQEGINILTHLPKGSAEAELMSVVPVFYVFHYLETGNHWNIFHSDPLIEKQKLKKKLKEGMLSIMSYRNADYSYS

SEQ ID NO: 9 - protein, 30 aa, Homo sapiens
SHKDMQLGRLHMKTLLPVSKPEIRSYFPES

SEQ ID NO: 10 - protein, 325 aa, Homo sapiens
SHKDMQLGRLHMKTLLPVSKPEIRSYFPESWLWEVHLVPRRKQLQFALPDSLTTWEIQGIGISNTGICVADTVKAKVFKDVFLEMNIPYSVVRGEQIQLKGTVYNYRTSGMQFCVKMSAVEGICTSESPVIDHQGTKSSKCVRQKVEGSSSHLVTFTVLPLEIGLHNINFSLETWFGKEILVKTLRVVPEGVKRESYSGVTLDPRGIYGTISRRKEFPYRIPLDLVPKTEIKRILSVKGLLVGEILSAVLSQEGINILTHLPKGSAEAELMSVVPVFYVFHYLETGNHWNIFHSDPLIEKQKLKKKLKEGMLSIMSYRNADYSYS

SEQ ID NO: 11 - protein, 17 aa, Homo sapiens
DHQGTKSSKCVRQKVEG

SEQ ID NO: 12 - protein, 74 aa, Homo sapiens
TLQKKIEEIAAKYKHSVVKKCCYDGACVNNDETCEQRAARISLGPRCIKAFTECCVVASQLRANISHKDMQLGR

SEQ ID NO: 13 - protein, 20 aa, Homo sapiens
CCYDGACVNNDETCEQRAAR

SEQ ID NO: 14 - protein, 18 aa, Homo sapiens
KCCYDGACVNNDETCEQR

SEQ ID NO: 15 - protein, 10 aa, Homo sapiens
VNNDETCEQR

SEQ ID NO: 16 - protein, 6 aa, Homo sapiens
VNNDET

SEQ ID NO: 17 - protein, 9 aa, Homo sapiens
AARISLGPR

SEQ ID NO: 18 - protein, 19 aa, Homo sapiens
CCYDGACVNNDETCEQRAA

SEQ ID NO: 19 - protein, 18 aa, Homo sapiens
CCYDGACVNNDETCEQRA

SEQ ID NO: 20 - protein, 17 aa, Homo sapiens
CCYDGACVNNDETCEQR

SEQ ID NO: 21 - protein, 16 aa, Homo sapiens
CCYDGACVNNDETCEQ

SEQ ID NO: 22 - protein, 15 aa, Homo sapiens
CCYDGACVNNDETCE

SEQ ID NO: 23 - protein, 19 aa, Homo sapiens
CYDGACVNNDETCEQRAAR

SEQ ID NO: 24 - protein, 18 aa, Homo sapiens
YDGACVNNDETCEQRAAR

SEQ ID NO: 25 - protein, 19 aa, Homo sapiens
CYDGACVNNDETCEQRAAR

SEQ ID NO: 26 - protein, 925 aa, Homo sapiens
LHMKTLLPVSKPEIRSYFPESWLWEVHLVPRRKQLQFALPDSLTTWEIQGIGISNTGICVADTVKAKVFKDVFLEMNIPYSVVRGEQIQLKGTVYNYRTSGMQFCVKMSAVEGICTSESPVIDHQGTKSSKCVRQKVEGSSSHLVTFTVLPLEIGLHNINFSLETWFGKEILVKTLRVVPEGVKRESYSGVTLDPRGIYGTISRRKEFPYRIPLDLVPKTEIKRILSVKGLLVGEILSAVLSQEGINILTHLPKGSAEAELMSVVPVFYVFHYLETGNHWNIFHSDPLIEKQKLKKKLKEGMLSIMSYRNADYSYSVWKGGSASTWLTAFALRVLGQVNKYVEQNQNSICNSLLWLVENYQLDNGSFKENSQYQPIKLQGTLPVEARENSLYLTAFTVIGIRKAFDICPLVKIDTALIKADNFLLENTLPAQSTFTLAISAYALSLGDKTHPQFRSIVSALKREALVKGNPPIYRFWKDNLQHKDSSVPNTGTARMVETTAYALLTSLNLKDINYVNPVIKWLSEEQRYGGGFYSTQDTINAIEGLTEYSLLVKQLRLSMDIDVSYKHKGALHNYKMTDKNFLGRPVEVLLNDDLIVSTGFGSGLATVHVTTVVHKTSTSEEVCSFYLKIDTQDIEASHYRGYGNSDYKRIVACASYKPSREESSSGSSHAVMDISLPTGISANEEDLKALVEGVDQLFTDYQIKDGHVILQLNSIPSSDFLCVRFRIFELFEVGFLSPATFTVYEYHRPDKQCTMFYSTSNIKIQKVCEGAACKCVEADCGQMQEELDLTISAETRKQTACKPEIAYAYKVSITSITVENVFVKYKATLLDIYKTGEAVAEKDSEITFIKKVTCTNAELVKGRQYLIMGKEALQIKYNFSFRYIYPLDSLTWIEYWPRDTTCSSCQAFLANLDEFAEDIFLNGC